European Patent Specification EP 3 639 008 B1, published March 1, 2023. Title: METHOD AND SYSTEM FOR ANALYSIS OF CRYSTALS AND CRYSTALLIZATION. Applicant: PROTEIN DYNAMIC SOLUTIONS LLC. The sequence listing filed with the application follows.

SEQUENCE LISTING (8 sequences)

SEQ ID NO: 1 - protein, 126 aa, Artificial Sequence
  Description of Artificial Sequence: Synthetic polypeptide
APELLGGPSVFLFPPKPKDTLMISRTPEVTCVVVDVSHEDPEVKFNWYVDGVEVHNAKTKPREEQYNSTYRVVSVLTVLHQDWLNGKEYKCKVSNKALPAPIEKTISKAKHHHHHHGDYKDDDDKG

SEQ ID NO: 2 - protein, 7 aa, Artificial Sequence
  Description of Artificial Sequence: Synthetic peptide
APELLGG

SEQ ID NO: 3 - protein, 119 aa, Artificial Sequence
  Description of Artificial Sequence: Synthetic polypeptide
PSVFLFPPKPKDTLMISRTPEVTCVVVDVSHEDPEVKFNWYVDGVEVHNAKTKPREEQYNSTYRVVSVLTVLHQDWLNGKEYKCKVSNKALPAPIEKTISKAKHHHHHHGDYKDDDDKG

SEQ ID NO: 4 - protein, 119 aa, Artificial Sequence
  Description of Artificial Sequence: Synthetic polypeptide
PSVFCFPPKPKDTLMISRTPEVTCVVVDVSHEDPEVKFNWYVDGVEVHNAKTKPREEQYNSTYRVVSVLTVLHQDWLNGKEYKCKVSNKALPAPIECTISKAKHHHHHHGDYKDDDDKG

SEQ ID NO: 5 - protein, 450 aa, Artificial Sequence
  Description of Artificial Sequence: Synthetic polypeptide
QVTLRESGPALVKPTQTLTLTCTFSGFSLSTAGMSVGWIRQPPGKALEWLADIWWDDKKHYNPSLKDRLTISKDTSKNQVVLKVTNMDPADTATYYCARDMIFNFYFDVWGQGTTVTVSSASTKGPSVFPLAPSSKSTSGGTAALGCLVKDYFPEPVTVSWNSGALTSGVHTFPAVLQSSGLYSLSSVVTVPSSSLGTQTYICNVNHKPSNTKVDKRVEPKSCDKTHTCPPCPAPELLGGPSVFLFPPKPKDTLMISRTPEVTCVVVDVSHEDPEVKFNWYVDGVEVHNAKTKPREEQYNSTYRVVSVLTVLHQDWLNGKEYKCKVSNKALPAPIEKTISKAKGQPREPQVYTLPPSREEMTKNQVSLTCLVKGFYPSDIAVEWESNGQPENNYKTTPPVLDSDGSFFLYSKLTVDKSRWQQGNVFSCSVMHEALHNHYTQKSLSLSPGK

SEQ ID NO: 6 - protein, 213 aa, Artificial Sequence
  Description of Artificial Sequence: Synthetic polypeptide
DIQMTQSPSTLSASVGDRVTITCSASSRVGYMHWYQQKPGKAPKLLIYDTSKLASGVPSRFSGSGSGTEFTLTISSLQPDDFATYYCFQGSGYPFTFGGGTKVEIKRTVAAPSVFIFPPSDEQLKSGTASVVCLLNNFYPREAKVQWKVDNALQSGNSQESVTEQDSKDSTYSLSSTLTLSKADYEKHKVYACEVTHQGLSSPVTKSFNRGEC

SEQ ID NO: 7 - protein, 583 aa, Bos taurus
DTHKSEIAHRFKDLGEEHFKGLVLIAFSQYLQQCPFDEHVKLVNELTEFAKTCVADESHAGCEKSLHTLFGDELCKVASLRETYGDMADCCEKQEPERNECFLSHKDDSPDLPKLKPDPNTLCDEFKADEKKFWGKYLYEIARRHPYFYAPELLYYANKYNGVFQECCQAEDKGACLLPKIETMREKVLTSSARQRLRCASIQKFGERALKAWSVARLSQKFPKAEFVEVTKLVTDLTKVHKECCHGDLLECADDRADLAKYICDNQDTISSKLKECCDKPLLEKSHCIAEVEKDAIPENLPPLTADFAEDKDVCKNYQEAKDAFLGSFLYEYSRRHPEYAVSVLLRLAKEYEATLEECCAKDDPHACYSTVFDKLKHLVDEPQNLIKQNCDQFEKLGEYGFQNALIVRYTRKVPQVSTPTLVEVSRSLGKVGTRCCTKPESERMPCTEDYLSLILNRLCVLHEKTPVSEKVTKCCTESLVNRRPCFSALTPDETYVPKAFDEKLFTFHADICTLPDTEKQIKKQTALVELLKHKPKATEEQLKTVMENFVAFVDKCCAADDKEACFAVEGPKLVVSTQTALA

SEQ ID NO: 8 - protein, 129 aa, Unknown [sequence omitted]